European Patent Specification EP 3 778 903 B1, published January 14, 2026. Title: TRI-SEGMENTED ARENAVIRUSES AS VACCINE VECTORS. Applicant: Université De Genève. Application to be assigned. The sequence listing filed with the application follows.

SEQUENCE LISTING (24 sequences)

SEQ ID NO: 1 - DNA, 3376 bp, Lymphocytic choriomeningitis virus (LCMV)
  cDNA sequence of LCMV segment S complete genomic sequence
cgcaccggggatcctaggctttttggattgcgctttcctctagatcaactgggtgtcaggccctatcctacagaaggatgggtcagattgtgacaatgtttgaggctctgcctcacatcatcgatgaggtgatcaacattgtcattattgtgcttatcgtgatcacgggtatcaaggctgtctacaattttgccacctgtgggatattcgcattgatcagtttcctacttctggctggcaggtcctgtggcatgtacggtcttaagggacccgacatttacaaaggagtttaccaatttaagtcagtggagtttgatatgtcacatctgaacctgaccatgcccaacgcatgttcagccaacaactcccaccattacatcagtatggggacttctggactagaattgaccttcaccaatgattccatcatcagtcacaacttttgcaatctgacctctgccttcaacaaaaagacctttgaccacacactcatgagtatagtttcgagcctacacctcagtatcagagggaactccaactataaggcagtatcctgcgacttcaacaatggcataaccatccaatacaacttgacattctcagatcgacaaagtgctcagagccagtgtagaaccttcagaggtagagtcctagatatgtttagaactgccttcggggggaaatacatgaggagtggctggggctggacaggctcagatggcaagaccacctggtgtagccagacgagttaccaatacctgattatacaaaatagaacctgggaaaaccactgcacatatgcaggtccttttgggatgtccaggattctcctttcccaagagaagactaagttcttcactaggagactagcgggcacattcacctggactttgtcagactcttcaggggtggagaatccaggtggttattgcctgaccaaatggatgattcttgctgcagagcttaagtgtttcgggaacacagcagttgcgaaatgcaatgtaaatcatgatgccgaattctgtgacatgctgcgactaattgactacaacaaggctgctttgagtaagttcaaagaggacgtagaatctgccttgcacttattcaaaacaacagtgaattctttgatttcagatcaactactgatgaggaaccacttgagagatctgatgggggtgccatattgcaattactcaaagttttggtacctagaacatgcaaagaccggcgaaactagtgtccccaagtgctggcttgtcaccaatggttcttacttaaatgagacccacttcagtgatcaaatcgaacaggaagccgataacatgattacagagatgttgaggaaggattacataaagaggcaggggagtacccccctagcattgatggaccttctgatgttttccacatctgcatatctagtcagcatcttcctgcaccttgtcaaaataccaacacacaggcacataaaaggtggctcatgtccaaagccacaccgattaaccaacaaaggaatttgtagttgtggtgcatttaaggtgcctggtgtaaaaaccgtctggaaaagacgctgaagaacagcgcctccctgactctccacctcgaaagaggtggagagtcagggaggcccagagggtcttagagtgtcacaacatttgggcctctaaaaattaggtcatgtggcagaatgttgtgaacagttttcagatctgggagccttgctttggaggcgctttcaaaaatgatgcagtccatgagtgcacagtgcggggtgatctctttcttctttttgtcccttactattccagtatgcatcttacacaaccagccatatttgtcccacactttgtcttcatactccctcgaagcttccctggtcatttcaacatcgataagcttaatgtccttcctattctgtgagtccagaagctttctgatgtcatcggagccttgacagcttagaaccatcccctgcggaagagcacctataactgacgaggtcaacccgggttgcgcattgaagaggtcggcaagatccatgccgtgtgagtacttggaatcttgcttgaattgtttttgatcaacgggttccctgtaaaagtgtatgaactgcccgttctgtggttggaaaattgctatttccactggatcattaaatctaccctcaatgtcaatccatgtaggagcgttggggtcaattcctcccatgaggtcttttaaaagcattgtctggctgtagcttaagcccacctgaggtggacctgctgctccaggcgctggcctgggtgaattgactgcaggtttctcgcttgtgagatcaattgttgtgttttcccatgctctccccacaatcgatgttctacaagctatgtatggccatccttcacctgaaaggcaaactttatagaggatgttttcataagggttcctgtccccaacttggtctgaaacaaacatgttgagttttctcttggccccgagaactgccttcaagaggtcctcgctgttgcttggcttgatcaaaattgactctaacatgttacccccatccaacagggctgcccctgccttcacggcagcaccaagactaaagttatagccagaaatgttgatgctggactgctgttcagtgatgacccccagaactgggtgcttgtctttcagcctttcaagatcattaagatttggatacttgactgtgtaaagcaagccaaggtctgtgagcgcttgtacaacgtcattgagcggagtctgtgactgtttggccatacaagccatagttagacttggcattgtgccaaattgattgttcaaaagtgatgagtctttcacatcccaaactcttaccacaccacttgcaccctgctgaggctttctcatcccaactatctgtaggatctgagatctttggtctagttgctgtgttgttaagttccccatatatacccctgaagcctggggcctttcagacctcatgatcttggccttcagcttctcaaggtcagccgcaagagacatcagttcttctgcactgagcctccccactttcaaaacattcttctttgatgttgactttaaatccacaagagaatgtacagtctggttgagacttctgagtctctgtaggtctttgtcatctctcttttccttcctcatgatcctctgaacattgctgacctcagagaagtccaacccattcagaaggttggttgcatccttaatgacagcagccttcacatctgatgtgaagctctgcaattctcttctcaatgcttgcgtccattggaagctcttaacttccttagacaaggacatcttgttgctcaatggtttctcaagacaaatgcgcaatcaaatgcctaggatccactgtgcg

SEQ ID NO: 2 - DNA, 3377 bp, Lymphocytic choriomeningitis virus (LCMV)
  LCMV clone 13 segment S complete sequence (GenBank: DQ361065.2)
gcgcaccggggatcctaggctttttggattgcgctttcctctagatcaactgggtgtcaggccctatcctacagaaggatgggtcagattgtgacaatgtttgaggctctgcctcacatcatcgatgaggtgatcaacattgtcattattgtgcttatcgtgatcacgggtatcaaggctgtctacaattttgccacctgtgggatattcgcattgatcagtttcctacttctggctggcaggtcctgtggcatgtacggtcttaagggacccgacatttacaaaggagtttaccaatttaagtcagtggagtttgatatgtcacatctgaacctgaccatgcccaacgcatgttcagccaacaactcccaccattacatcagtatggggacttctggactagaattgaccttcaccaatgattccatcatcagtcacaacttttgcaatctgacctctgccttcaacaaaaagacctttgaccacacactcatgagtatagtttcgagcctacacctcagtatcagagggaactccaactataaggcagtatcctgcgacttcaacaatggcataaccatccaatacaacttgacattctcagatgcacaaagtgctcagagccagtgtagaaccttcagaggtagagtcctagatatgtttagaactgccttcggggggaaatacatgaggagtggctggggctggacaggctcagatggcaagaccacctggtgtagccagacgagttaccaatacctgattatacaaaatagaacctgggaaaaccactgcacatatgcaggtccttttgggatgtccaggattctcctttcccaagagaagactaagttcctcactaggagactagcgggcacattcacctggactttgtcagactcttcaggggtggagaatccaggtggttattgcctgaccaaatggatgattcttgctgcagagcttaagtgtttcgggaacacagcagttgcgaaatgcaatgtaaatcatgatgaagaattctgtgacatgctgcgactaattgactacaacaaggctgctttgagtaagttcaaagaggacgtagaatctgccttgcacttattcaaaacaacagtgaattctttgatttcagatcaactactgatgaggaaccacttgagagatctgatgggggtgccatattgcaattactcaaagttttggtacctagaacatgcaaagaccggcgaaactagtgtccccaagtgctggcttgtcaccaatggttcttacttaaatgagacccacttcagtgaccaaatcgaacaggaagccgataacatgattacagagatgttgaggaaggattacataaagaggcaggggagtacccccctagcattgatggaccttctgatgttttccacatctgcatatctagtcagcatcttcctgcaccttgtcaaaataccaacacacaggcacataaaaggtggctcatgtccaaagccacaccgattaaccaacaaaggaatttgtagttgtggtgcatttaaggtgcctggtgtaaaaaccgtctggaaaagacgctgaagaacagcgcctccctgactctccacctcgaaagaggtggagagtcagggaggcccagagggtcttagagtgtcacaacatttgggcctctaaaaattaggtcatgtggcagaatgttgtgaacagttttcagatctgggagccttgctttggaggcgctttcaaaaatgatgcagtccatgagtgcacagtgcggggtgatctctttcttctttttgtcccttactattccagtatgcatcttacacaaccagccatatttgtcccacactttgtcttcatactccctcgaagcttccctggtcatttcaacatcgataagcttaatgtccttcctattctgtgagtccagaagctttctgatgtcatcggagccttgacagcttagaaccatcccctgcggaagagcacctataactgacgaggtcaacccgggttgcgcattgaagaggtcggcaagatccatgccgtgtgagtacttggaatcttgcttgaattgtttttgatcaacgggttccctgtaaaagtgtatgaactgcccgttctgtggttggaaaattgctatttccactggatcattaaatctaccctcaatgtcaatccatgtaggagcgttggggtcaattcctcccatgaggtcttttaaaagcattgtctggctgtagcttaagcccacctgaggtggacctgctgctccaggcgctggcctgggtgaattgactgcaggtttctcgcttgtgagatcaattgttgtgttttcccatgctctccccacaatcgatgttctacaagctatgtatggccatccttcacctgaaaggcaaactttatagaggatgttttcataagggttcctgtccccaacttggtctgaaacaaacatgttgagttttctcttggccccgagaactgccttcaagaggtcctcgctgttgcttggcttgatcaaaattgactctaacatgttacccccatccaacagggctgcccctgccttcacggcagcaccaagactaaagttatagccagaaatgttgatgctggactgctgttcagtgatgacccccagaactgggtgcttgtctttcagcctttcaagatcattaagatttggatacttgactgtgtaaagcaagccaaggtctgtgagcgcttgtacaacgtcattgagcggagtctgtgactgtttggccatacaagccatagttagacttggcattgtgccaaattgattgttcaaaagtgatgagtctttcacatcccaaactcttaccacaccacttgcaccctgctgaggctttctcatcccaactatctgtaggatctgagatctttggtctagttgctgtgttgttaagttccccatatatacccctgaagcctggggcctttcagacctcatgatcttggccttcagcttctcaaggtcagccgcaagagacatcagttcttctgcactgagcctccccactttcaaaacattcttctttgatgttgactttaaatccacaagagaatgtacagtctggttgagacttctgagtctctgtaggtctttgtcatctctcttttccttcctcatgatcctctgaacattgctgacctcagagaagtccaacccattcagaaggttggttgcatccttaatgacagcagccttcacatctgatgtgaagctctgcaattctcttctcaatgcttgcgtccattggaagctcttaacttccttagacaaggacatcttgttgctcaatggtttctcaagacaaatgcgcaatcaaatgcctaggatccactgtgcg

SEQ ID NO: 3 - DNA, 7229 bp, Lymphocytic choriomeningitis virus (LCMV)
  LCMV clone 13 segment L complete sequence (GenBank: DQ361066.1)
gcgcaccggggatcctaggcgtttagttgcgctgtttggttgcacaactttcttcgtgaggctgtcagaagtggacctggctgatagcgatgggtcaaggcaagtccagagaggagaaaggcaccaatagtacaaacagggccgaaatcctaccagataccacctatcttggccctttaagctgcaaatcttgctggcagaaatttgacagcttggtaagatgccatgaccactacctttgcaggcactgtttaaaccttctgctgtcagtatccgacaggtgtcctctttgtaaatatccattaccaaccagattgaagatatcaacagccccaagctctccacctccctacgaagagtaacaccgtccggccccggccccgacaaacagcccagcacaagggaaccgcacgtcacccaacgcacacagacacagcacccaacacagaacacgcacacacacacacacacacacccacacgcacgcgcccccaccaccggggggcgcccccccccggggggcggccccccgggagcccgggcggagccccacggagatgcccatcagtcgatgtcctcggccaccgacccgcccagccaatcgtcgcaggacctccccttgagtctaaacctgccccccactgtttcatacatcaaagtgctcctagatttgctaaaacaaagtctgcaatccttaaaggcgaaccagtctggcaaaagcgacagtggaatcagcagaatagatctgtctatacatagttcctggaggattacacttatctctgaacccaacaaatgttcaccagttctgaatcgatgcaggaagaggttcccaaggacatcactaatcttttcatagccctcaagtcctgctagaaagactttcatgtccttggtctccagcttcacaatgatattttggacaaggtttcttccttcaaaaagggcacccatctttacagtcagtggcacaggctcccactcaggtccaactctctcaaagtcaatagatctaatcccatccagtattcttttggagcccaacaactcaagctcaagagaatcaccaagtatcaagggatcttccatgtaatcctcaaactcttcagatctgatatcaaagacaccatcgttcaccttgaagacagagtctgtcctcagtaagtggaggcattcatccaacattcttctatctatctcacccttaaagaggtgagagcatgataaaagttcagccacacctggattctgtaattggcacctaaccaagaatatcaatgaaaatttccttaaacagtcagtattattctgattgtgcgtaaagtccactgaaattgaaaactccaataccccttttgtgtagttgagcatgtagtcccacagatcctttaaggatttaaatgcctttgggtttgtcaggccctgcctaatcaacatggcagcattacacacaacatctcccattcggtaagagaaccacccaaaaccaaactgcaaatcattcctaaacataggcctctccacatttttgttcaccacctttgagacaaatgattgaaaggggcccagtgcctcagcaccatcttcagatggcatcatttctttatgagggaaccatgaaaaattgcctaatgtcctggttgttgcaacaaattctcgaacaaatgattcaaaatacacctgttttaagaagttcttgcagacatccctcgtgctaacaacaaattcatcaaccagactggagtcagatcgctgatgagaattggcaaggtcagaaaacagaacagtgtaatgttcatcccttttccacttaacaacatgagaaatgagtgacaaggattctgagttaatatcaattaaaacacagaggtcaaggaatttaattctgggactccacctcatgttttttgagctcatgtcagacataaatggaagaagctgatcctcaaagatcttgggatatagccgcctcacagattgaatcacttggttcaaattcactttgtcctccagtagccttgagctctcaggctttcttgctacataatcacatgggtttaagtgcttaagagttaggttctcactgttattcttccctttggtcggttctgctaggacccaaacacccaactcaaaagagttgctcaatgaaatacaaatgtagtcccaaagaagaggccttaaaaggcatatatgatcacggtgggcttctggatgagactgtttgtcacaaatgtacagcgttataccatcccgattgcaaactcttgtcacatgatcatctgtggttagatcctcaagcagctttttgatatacagattttccctatttttgtttctcacacacctgcttcctagagttttgcaaaggcctataaagccagatgagatacaactctggaaagctgacttgttgattgcttctgacagcagcttctgtgcaccccttgtgaatttactacaaagtttgttctggagtgtcttgatcaatgatgggattctttcctcttggaaagtcatcactgatggataaaccaccttttgtcttaaaaccatccttaatgggaacatttcattcaaattcaaccagttaacatctgctaactgattcagatcttcttcaagaccgaggaggtctcccaattgaagaatggcctcctttttatctctgttaaataggtctaagaaaaattcttcattaaattcaccatttttgagcttatgatgcagtttccttacaagctttcttacaacctttgtttcattaggacacagttcctcaatgagtctttgtattctgtaacctctagaaccatccagccaatctttcacatcagtgttggtattcagtagaaatggatccaaagggaaattggcatactttaggaggtccagtgttctcctttggatactattaactagggagactgggacgccatttgcgatggcttgatctgcaattgtatctattgtttcacaaagttgatgtggctctttacacttgacattgtgtagcgctgcagatacaaactttgtgagaagagggacttcctccccccatacatagaatctagatttaaattctgcagcgaacctcccagccacactttttgggctgataaatttgtttaacaagccgctcagatgagattggaattccaacaggacaaggacttcctccggatcacttacaaccaggtcactcagcctcctatcaaataaagtgatctgatcatcacttgatgtgtaagcctctggtctttcgccaaagataacaccaatgcagtagttgatgaacctctcgctaagcaaaccatagaagtcagaagcattatgcaagattccctgccccatatcaataaggctggatatatgggatggcactatccccatttcaaaatattgtctgaaaattctctcagtaacagttgtttctgaacccctgagaagttttagcttcgacttgacatatgatttcatcattgcattcacaacaggaaaggggacctcgacaagcttatgcatgtgccaagttaacaaagtgctaacatgatctttcccggaacgcacatactggtcatcacctagtttgagattttgtagaaacattaagaacaaaaatgggcacatcattggtccccatttgctgtgatccatactatagtttaagaacccttcccgcacattgatagtcattgacaagattgcattttcaaattccttatcattgtttaaacaggagcctgaaaagaaacttgaaaaagactcaaaataatcttctattaaccttgtgaacatttttgtcctcaaatctccaatatagagttctctatttcccccaacctgctctttataagatagtgcaaatttcagccttccagagtcaggacctactgaggtgtatgatgttggtgattcttctgagtagaagcacagatttttcaaagcagcactcatacattgtgtcaacgacagagctttactaagggactcagaattactttccctctcactgattctcacgtcttcttccagtttgtcccagtcaaatttgaaattcaagccttgcctttgcatatgcctgtatttccctgagtacgcatttgcattcatttgcaacagaatcatcttcatgcaagaaaaccaatcattctcagaaaagaactttctacaaaggttttttgccatctcatcgaggccacactgatctttaatgactgaggtgaaatacaaaggtgacagctctgtggaaccctcaacagcctcacagataaatttcatgtcatcattggttagacatgatgggtcaaagtcttctactaaatggaaagatatttctgacaagataacttttcttaagtgagccatcttccctgttagaataagctgtaaatgatgtagtccttttgtatttgtaagtttttctccatctcctttgtcattggccctcctacctcttctgtaccgtgctattgtggtgttgaccttttcttcgagacttttgaagaagcttgtctcttcttctccatcaaaacatatttctgccaggttgtcttccgatctccctgtctcttctcccttggaaccgatgaccaatctagagactaacttggaaactttatattcatagtctgagtggctcaacttatacttttgttttcttacgaaactctccgtaatttgactcacagcactaacaagcaatttgttaaagtcatattccagaagtcgttctccatttagatgcttattaaccaccacacttttgttactagcaagatctaatgctgtcgcacatccagagttagtcatgggatctaggctgtttagcttcttctctcctttgaaaattaaagtgccgttgttaaatgaagacaccattaggctaaaggcttccagattaacacctggagttgtatgctgacagtcaatttctttactagtgaatctcttcatttgctcatagaacacacattcttcctcaggagtgattgcttccttggggttgacaaaaaaaccaaattgacttttgggctcaaagaacttttcaaaacattttatctgatctgttagcctgtcaggggtctcctttgtgatcaaatgacacaggtatgacacattcaacataaatttaaattttgcactcaacaacaccttctcaccagtaccaaaaatagtttttattaggaatctaagcagcttatacaccaccttctcagcaggtgtgatcagatcctccctcaacttatccattaatgatgtagatgaaaaatctgacactattgccatcaccaaatatctgacactctgtacctgcttttgatttctctttgttgggttggtgagcattagcaacaatagggtcctcagtgcaacctcaatgtcggtgagacagtctttcaaatcaggacatgatctaatccatgaaatcatgatgtctatcatattgtataagacctcatctgaaaaaattggtaaaaagaaccttttaggatctgcatagaaggaaattaaatgaccatccgggccttgtatggagtagcaccttgaagattctccagtcttctggtataataggtggtattcttcagagtccagttttattacttggcaaaacacttctttgcattctaccacttgatatctcacagaccctatttgattttgccttagtctagcaactgagctagttttcatactgtttgttaaggccagacaaacagatgataatcttctcaggctctgtatgttcttcagctgctctgtgctgggttggaaattgtaatcttcaaacttcgtataatacattatcgggtgagctccaattttcataaagttctcaaattcagtgaatggtatgtggcattcttgctcaaggtgttcagacagtccgtaatgctcgaaactcagtcccaccactaacaggcatttttgaatttttgcaatgaactcactaatagatgccctaaacaattcctcaaaagacacctttctaaacacctttgacttttttctattcctcaaaagtctaatgaactcctctttagtgctgtgaaagcttaccagcctatcattcacactactatagcaacaacccacccagtgtttatcattttttaaccctttgaatttcgactgttttatcaatgaggaaagacacaaaacatccagatttaacaactgtctccttctagtattcaacagtttcaaactcttgactttgtttaacatagagaggagcctctcatattcagtgctagtctcacttcccctttcgtgcccatgggtctctgcagttatgaatctcatcaaaggacaggattcgactgcctccctgcttaatgttaagatatcatcactatcagcaaggttttcatagagctcagagaattccttgatcaagccttcagggtttactttctgaaagtttctctttaatttcccactttctaaatctcttctaaacctgctgaaaagagagtttattccaaaaaccacatcatcacagctcatgttggggttgatgccttcgtggcacatcctcataatttcatcattgtgagttgacctcgcatctttcagaattttcatagagtccataccggagcgcttgtcgatagtagtcttcagggactcacagagtctaaaatattcagactcttcaaagactttctcattttggttagaatactccaaaagtttgaataaaaggtctctaaatttgaagtttgcccactctggcataaaactattatcataatcacaacgaccatctactattggaactaatgtgacacccgcaacagcaaggtcttccctgatgcatgccaatttgttagtgtcctctataaatttcttctcaaaactggctggagtgctcctaacaaaacactcaagaagaatgagagaattgtctatcagcttgtaaccatcaggaatgataagtggtagtcctgggcatacaattccagactccaccaaaattgtttccacagacttatcgtcgtggttgtgtgtgcagccactcttgtctgcactgtctatttcaatgcagcgtgacagcaacttgagtccctcaatcagaaccattctgggttccctttgtcccagaaagttgagtttctgccttgacaacctctcatcctgttctatatagtttaaacataactctctcaattctgagatgatttcatccattgcgcatcaaaaagcctaggatcctcggtgcg

SEQ ID NO: 4 - DNA, 7205 bp, Lymphocytic choriomeningitis virus (LCMV)
  LCMV strain MP segment L complete sequence
gcgcaccggggatcctaggcatttttgttgcgcattttgttgtgttatttgttgcacagcccttcatcgtgggaccttcacaaacaaaccaaaccaccagccatgggccaaggcaagtccaaagagggaagggatgccagcaatacgagcagagctgaaattctgccagacaccacctatctcggacctctgaactgcaagtcatgctggcagagatttgacagtttagtcagatgccatgaccactatctctgcagacactgcctgaacctcctgctgtcagtctccgacaggtgccctctctgcaaacatccattgccaaccaaactgaaaatatccacggccccaagctctccacccccttacgaggagtgacgccccgagccccaacaccgacacaaggaggccaccaacacaacgcccaacacggaacacacacacacacacccacacacacatccacacacacgcgcccccacaacgggggcgcccccccgggggtggccccccgggtgctcgggcggagccccacggagaggccaattagtcgatctcctcgaccaccgacttggtcagccagtcatcacaggacttgcccttaagtctgtacttgcccacaactgtttcatacatcaccgtgttctttgacttactgaaacatagcctacagtctttgaaagtgaaccagtcaggcacaagtgacagcggtaccagtagaatggatctatctatacacaactcttggagaattgtgctaatttccgacccctgtagatgctcaccagttctgaatcgatgtagaagaaggctcccaaggacgtcatcaaaatttccataaccctcgagctctgccaagaaaactctcatatccttggtctccagtttcacaacgatgttctgaacaaggcttcttccctcaaaaagagcacccattctcacagtcaagggcacaggctcccattcaggcccaatcctctcaaaatcaagggatctgatcccgtccagtattttccttgagcctatcagctcaagctcaagagagtcaccgagtatcagggggtcctccatatagtcctcaaactcttcagacctaatgtcaaaaacaccatcgttcaccttgaagatagagtctgatctcaacaggtggaggcattcgtccaagaaccttctgtccacctcacctttaaagaggtgagagcatgataggaactcagctacacctggaccttgtaactggcacttcactaaaaagatcaatgaaaacttcctcaaacaatcagtgttattctggttgtgagtgaaatctactgtaattgagaactctagcactccctctgtattatttatcatgtaatcccacaagtttctcaaagacttgaatgcctttggatttgtcaagccttgtttgattagcatggcagcattgcacacaatatctcccaatcggtaagagaaccatccaaatccaaattgcaagtcattcctaaacatgggcctctccatatttttgttcactacttttaagatgaatgattggaaaggccccaatgcttcagcgccatcttcagatggcatcatgtctttatgagggaaccatgaaaaacttcctagagttctgcttgttgctacaaattctcgtacaaatgactcaaaatacacttgttttaaaaagtttttgcagacatcccttgtactaacgacaaattcatcaacaaggcttgagtcagagcgctgatgggaatttacaagatcagaaaatagaacagtgtagtgttcgtccctcttccacttaactacatgagaaatgagcgataaagattctgaattgatatcgatcaatacgcaaaggtcaaggaatttgattctgggactccatctcatgttttttgagctcatatcagacatgaagggaagcagctgatcttcatagattttagggtacaatcgcctcacagattggattacatggtttaaacttatcttgtcctccagtagccttgaactctcaggcttccttgctacataatcacatgggttcaagtgcttgaggcttgagcttccctcattcttccctttcacaggttcagctaagacccaaacacccaactcaaaggaattactcagtgagatgcaaatatagtcccaaaggaggggcctcaagagactgatgtggtcgcagtgagcttctggatgactttgcctgtcacaaatgtacaacattatgccatcatgtctgtggattgctgtcacatgcgcatccatagctagatcctcaagcacttttctaatgtatagattgtccctatttttatttctcacacatctacttcccaaagttttgcaaagacctataaagcctgatgagatgcaactttgaaaggctgacttattgattgcttctgacagcaacttctgtgcacctcttgtgaacttactgcagagcttgttctggagtgtcttgattaatgatgggattctttcctcttggaaagtcattactgatggataaaccactttctgcctcaagaccattcttaatgggaacaactcattcaaattcagccaatttatgtttgccaattgacttagatcctcttcgaggccaaggatgtttcccaactgaagaatggcttcctttttatccctattgaagaggtctaagaagaattcttcattgaactcaccattcttgagcttatgatgtagtctccttacaagccttctcatgaccttcgtttcactaggacacaattcttcaataagcctttggattctgtaacctctagagccatccaaccaatccttgacatcagtattagtgttaagcaaaaatgggtccaagggaaagttggcatattttaagaggtctaatgttctcttctggatgcagtttaccaatgaaactggaacaccatttgcaacagcttgatcggcaattgtatctattgtttcacagagttggtgtggctctttacacttaacgttgtgtaatgctgctgacacaaattttgttaaaagtgggacctcttccccccacacataaaatctggatttaaattctgcagcaaatcgccccaccacacttttcggactgatgaacttgttaagcaagccactcaaatgagaatgaaattccagcaatacaaggacttcctcagggtcactatcaaccagttcactcaatctcctatcaaataaggtgatctgatcatcacttgatgtgtaagattctggtctctcaccaaaaatgacaccgatacaataattaatgaatctctcactgattaagccgtaaaagtcagaggcattatgtaagattccctgtcccatgtcaatgagactgcttatatgggaaggcactattcctaattcaaaatattctcgaaagattctttcagtcacagttgtctctgaacccctaagaagtttcagctttgatttgatatatgatttcatcattgcattcacaacaggaaaagggacctcaacaagtttgtgcatgtgccaagttaataaggtgctgatatgatcctttccggaacgcacatactggtcatcacccagtttgagattttgaaggagcattaaaaacaaaaatgggcacatcattggcccccatttgctatgatccatactgtagttcaacaacccctctcgcacattgatggtcattgatagaattgcattttcaaattctttgtcattgtttaagcatgaacctgagaagaagctagaaaaagactcaaaataatcctctatcaatcttgtaaacatttttgttctcaaatccccaatataaagttctctgtttcctccaacctgctctttgtatgataacgcaaacttcaaccttccggaatcaggaccaactgaagtgtatgacgttggtgactcctctgagtaaaaacataaattctttaaagcagcactcatgcattttgtcaatgatagagccttacttagagactcagaattactttccctttcactaattctaacatcttcttctagtttgtcccagtcaaacttgaaattcagaccttgtctttgcatgtgcctgtatttccctgagtatgcatttgcattcatttgcagtagaatcattttcatacacgaaaaccaatcaccctctgaaaaaaacttcctgcagaggttttttgccatttcatccagaccacattgttctttgacagctgaagtgaaatacaatggtgacagttctgtagaagtttcaatagcctcacagataaatttcatgtcatcattggtgagacaagatgggtcaaaatcttccacaagatgaaaagaaatttctgataagatgaccttccttaaatatgccattttacctgacaatatagtctgaaggtgatgcaatccttttgtattttcaaaccccacctcattttccccttcattggtcttcttgcttctttcataccgctttattgtggagttgaccttatcttctaaattcttgaagaaacttgtctcttcttccccatcaaagcatatgtctgctgagtcaccttctagtttcccagcttctgtttctttagagccgataaccaatctagagaccaactttgaaaccttgtactcgtaatctgagtggttcaatttgtacttctgctttctcatgaagctctctgtgatctgactcacagcactaacaagcaatttgttaaaatcatactctaggagccgttccccatttaaatgtttgttaacaaccacacttttgttgctggcaaggtctaatgctgttgcacacccagagttagtcatgggatccaagctattgagcctcttctcccctttgaaaatcaaagtgccattgttgaatgaggacaccatcatgctaaaggcctccagattgacacctggggttgtgcgctgacagtcaacttctttcccagtgaacttcttcatttggtcataaaaaacacactcttcctcaggggtgattgactctttagggttaacaaagaagccaaactcacttttaggctcaaagaatttctcaaagcatttaatttgatctgtcagcctatcaggggtttcctttgtgattaaatgacacaggtatgacacattcaacatgaacttgaactttgcgctcaacagtaccttttcaccagtcccaaaaacagttttgatcaaaaatctgagcaatttgtacactactttctcagcaggtgtgatcaaatcctccttcaacttgtccatcaatgatgtggatgagaagtctgagacaatggccatcactaaatacctaatgttttgaacctgtttttgattcctctttgttgggttggtgagcatgagtaataatagggttctcaatgcaatctcaacatcatcaatgctgtccttcaagtcaggacatgatctgatccatgagatcatggtgtcaatcatgttgtgcaacacttcatctgagaagattggtaaaaagaacctttttgggtctgcataaaaagagattagatggccattgggaccttgtatagaataacaccttgaggattctccagtcttttgatacagcaggtgatattcctcagagtccaattttatcacttggcaaaatacctctttacattccaccacttgataccttacagagcccaattggttttgtcttaatctagcaactgaacttgttttcatactgtttgtcaaagctagacagacagatgacaatcttttcaaactatgcatgttccttaattgttccgtattaggctggaaatcataatcttcaaactttgtataatacattataggatgagttccggacctcatgaaattctcaaactcaataaatggtatgtggcactcatgctcaagatgttcagacagaccatagtgcccaaaactaagtcccaccactgacaagcacctttgaacttttaaaatgaactcatttatggatgttctaaacaaatcctcaagagatacctttctatacgcctttgactttctcctgttccttagaagtctgatgaactcttccttggtgctatgaaagctcaccaacctatcattcacactcccatagcaacaaccaacccagtgcttatcattttttgaccctttgagtttagactgtttgatcaacgaagagagacacaagacatccaaattcagtaactgtctccttctggtgttcaataattttaaacttttaactttgttcaacatagagaggagcctctcatactcagtgctagtctcacttcctctctcataaccatgggtatctgctgtgataaatctcatcaaaggacaggattcaactgcctccttgcttagtgctgaaatgtcatcactgtcagcaagagtctcataaagctcagagaattccttaattaaatttccggggttgattttctgaaaactcctcttgagcttcccagtttccaagtctcttctaaacctgctgtaaagggagtttatgccaagaaccacatcatcgcagttcatgtttgggttgacaccatcatggcacattttcataatttcatcattgtgaaatgatcttgcatctttcaagattttcatagagtctataccggaacgcttatcaacagtggtcttgagagattcgcaaagtctgaagtactcagattcctcaaagactttctcatcttggctagaatactctaaaagtttaaacagaaggtctctgaacttgaaattcacccactctggcataaagctgttatcataatcacaccgaccatccactattgggaccaatgtgatacccgcaatggcaaggtcttctttgatacaggctagtttattggtgtcctctataaatttcttctcaaaactagctggtgtgcttctaacgaagcactcaagaagaatgagggaattgtcaatcagtttataaccatcaggaatgatcaaaggcagtcccgggcacacaatcccagactctattagaattgcctcaacagatttatcatcatggttgtgtatgcagccgctcttgtcagcactgtctatctctatacaacgcgacaaaagtttgagtccctctatcaataccattctgggttctctttgccctaaaaagttgagcttctgccttgacaacctctcatcttgttctatgtggtttaagcacaactctctcaactccgaaatagcctcatccattgcgcatcaaaaagcctaggatcctcggtgcg

SEQ ID NO: 5 - DNA, 3359 bp, Lymphocytic choriomeningitis virus (LCMV)
  LCMV strain MP segment S complete sequence
cgcaccggggatcctaggctttttggattgcgctttcctcagctccgtcttgtgggagaatgggtcaaattgtgacgatgtttgaggctctgcctcacatcattgatgaggtcattaacattgtcattatcgtgcttattatcatcacgagcatcaaagctgtgtacaatttcgccacctgcgggatacttgcattgatcagctttctttttctggctggcaggtcctgtggaatgtatggtcttgatgggcctgacatttacaaaggggtttaccgattcaagtcagtggagtttgacatgtcttaccttaacctgacgatgcccaatgcatgttcggcaaacaactcccatcattatataagtatggggacttctggattggagttaaccttcacaaatgactccatcatcacccacaacttttgtaatctgacttccgccctcaacaagaggacttttgaccacacacttatgagtatagtctcaagtctgcacctcagcattagaggggtccccagctacaaagcagtgtcctgtgattttaacaatggcatcactattcaatacaacctgtcattttctaatgcacagagcgctctgagtcaatgtaagaccttcagggggagagtcctggatatgttcagaactgcttttggaggaaagtacatgaggagtggctggggctggacaggttcagatggcaagactacttggtgcagccagacaaactaccaatatctgattatacaaaacaggacttgggaaaaccactgcaggtacgcaggccctttcggaatgtctagaattctcttcgctcaagaaaagacaaggtttctaactagaaggcttgcaggcacattcacttggactttatcagactcatcaggagtggagaatccaggtggttactgcttgaccaagtggatgatcctcgctgcagagctcaagtgttttgggaacacagctgttgcaaagtgcaatgtaaatcatgatgaagagttctgtgatatgctacgactgattgattacaacaaggctgctttgagtaaattcaaagaagatgtagaatccgctctacatctgttcaagacaacagtgaattctttgatttctgatcagcttttgatgagaaatcacctaagagacttgatgggagtgccatactgcaattactcgaaattctggtatctagagcatgcaaagactggtgagactagtgtccccaagtgctggcttgtcagcaatggttcttatttgaatgaaacccatttcagcgaccaaattgagcaggaagcagataatatgatcacagaaatgctgagaaaggactacataaaaaggcaagggagtacccctctagccttgatggatctattgatgttttctacatcagcatatttgatcagcatctttctgcatcttgtgaggataccaacacacagacacataaagggcggctcatgcccaaaaccacatcggttaaccagcaagggaatctgtagttgtggtgcatttaaagtaccaggtgtggaaaccacctggaaaagacgctgaacagcagcgcctccctgactcaccacctcgaaagaggtggtgagtcagggaggcccagagggtcttagagtgttacgacatttggacctctgaagattaggtcatgtggtaggatattgtggacagttttcaggtcggggagccttgccttggaggcgctttcaaagatgatacagtccatgagtgcacagtgtggggtgacctctttctttttcttgtccctcactattccagtgtgcatcttgcatagccagccatatttgtcccagactttgtcctcatattctcttgaagcttctttagtcatctcaacatcgatgagcttaatgtctcttctgttttgtgaatctaggagtttcctgatgtcatcagatccctgacaacttaggaccattccctgtggaagagcacctattactgaagatgtcagcccaggttgtgcattgaagaggtcagcaaggtccatgccatgtgagtatttggagtcctgcttgaattgtttttgatcagtgggttctctatagaaatgtatgtactgcccattctgtggctgaaatattgctatttctaccgggtcattaaatctgccctcaatgtcaatccatgtaggagcgttagggtcaatacctcccatgaggtccttcagcaacattgtttggctgtagcttaagcccacctgaggtgggcccgctgccccaggcgctggtttgggtgagttggccataggcctctcatttgtcagatcaattgttgtgttctcccatgctctccctacaactgatgttctacaagctatgtatggccacccctcccctgaaagacagactttgtagaggatgttctcgtaaggattcctgtctccaacctgatcagaaacaaacatgttgagtttcttcttggccccaagaactgctttcaggagatcctcactgttgcttggcttaattaagatggattccaacatgttacccccatctaacaaggctgcccctgctttcacagcagcaccgagactgaaattgtagccagatatgttgatgctagactgctgctcagtgatgactcccaagactgggtgcttgtctttcagcctttcaaggtcacttaggttcgggtacttgactgtgtaaagcagcccaaggtctgtgagtgcttgcacaacgtcattgagtgaggtttgtgattgtttggccatacaagccattgttaagcttggcattgtgccgaattgattgttcagaagtgatgagtccttcacatcccagaccctcaccacaccatttgcactctgctgaggtctcctcattccaaccatttgcagaatctgagatctttggtcaagctgttgtgctgttaagttccccatgtagactccagaagttagaggcctttcagacctcatgattttagccttcagtttttcaaggtcagctgcaagggacatcagttcttctgcactaagcctccctacttttagaacattcttttttgatgttgactttaggtccacaagggaatacacagtttggttgaggcttctgagtctctgtaaatctttgtcatccctcttctctttcctcatgatcctctgaacattgctcacctcagagaagtctaatccattcagaaggctggtggcatccttgatcacagcagctttcacatctgatgtgaagccttgaagctctctcctcaatgcctgggtccattgaaagcttttaacttctttggacagagacattttgtcactcagtggatttccaagtcaaatgcgcaatcaaaatgcctaggatccactgtgcg

SEQ ID NO: 6 - protein, 552 aa, Lymphocytic choriomeningitis virus (LCMV)
  Amino acid sequence of the NP protein of the MP strain of LCMV
MSLSKEVKSFQWTQALRRELQGFTSDVKAAVIKDATSLLNGLDFSEVSNVQRIMRKEKRDDKDLQRLRSLNQTVYSLVDLKSTSKKNVLKVGRLSAEELMSLAADLEKLKAKIMRSERPLTSGVYMGNLTAQQLDQRSQILQMVGMRRPQQSANGVVRVWDVKDSSLLNNQFGTMPSLTMACMAKQSQTSLNDVVQALTDLGLLYTVKYPNLSDLERLKDKHPVLGVITEQQSSINISGYNFSLGAAVKAGAALLDGGNMLESILIKPSNSEDLLKAVLGAKKKLNMFDRNPYENILYKVCLSGEGWPYIACRTSVVGRAWENTTIDLTNERPMANSPKPAPGAAGPPQVGLSYSQTMLLKDLMGGIDPNAPTWIDIEGRFNDPVEIAIFQPQNGQYIHFYREPTDQKQFKQDSKYSHGMDLADLFNAQPGLTSSVIGALPQGMVLSCQGSDDIRKLLDSQNRRDIKLIDVEMTKEASREYEDKVWDKYGWLCKMHTGIVRDKKKKEVTPHCALMDCIIFESASKARLPDLKTVHNILPHDLIFRGPNVVTL

SEQ ID NO: 7 - protein, 498 aa, Lymphocytic choriomeningitis virus (LCMV)
  Amino acid sequence of the GP protein of the MP strain of LCMV
MGQIVTMFEALPHIIDEVINIVIIVLIIITSIKAVYNFATCGILALISFLFLAGRSCGMYGLDGPDIYKGVYRFKSVEFDMSYLNLTMPNACSANNSHHYISMGTSGLELTFTNDSIITHNFCNLTSALNKRTFDHTLMSIVSSLHLSIRGVPSYKAVSCDFNNGITIQYNLSFSNAQSALSQCKTFRGRVLDMFRTAFGGKYMRSGWGWTGSDGKTTWCSQTNYQYLIIQNRTWENHCRYAGPFGMSRILFAQEKTRFLTRRLAGTFTWTLSDSSGVENPGGYCLTKWMILAAELKCFGNTAVAKCNVNHDEEFCDMLRLIDYNKAALSKFKEDVESALHLFKTTVNSLISDQLLMRNHLRDLMGVPYCNYSKFWYLEHAKTGETSVPKCWLVSNGSYLNETHFSDQIEQEADNMITEMLRKDYIKRQGSTPLALMDLLMFSTSAYLISIFLHLVRIPTHRHIKGGSCPKPHRLTSKGICSCGAFKVPGVETTWKRR

SEQ ID NO: 8 - protein, 2201 aa, Lymphocytic choriomeningitis virus (LCMV)
  Amino acid sequence of the L protein of the MP strain of LCMV
MDEAISELRELCLNHIEQDERLSRQKLNFLGQREPRMVLIEGLKLLSRCIEIDSADKSGCIHNHDDKSVEAILIESGIVCPGLPLIIPDGYKLIDNSLILLECFVRSTPASFEKKFIEDTNKLACIKEDLAIAGITLVPIVDGRCDYDNSFMPEWVNFKFRDLLFKLLEYSSQDEKVFEESEYFRLCESLKTTVDKRSGIDSMKILKDARSFHNDEIMKMCHDGVNPNMNCDDVVLGINSLYSRFRRDLETGKLKRSFQKINPGNLIKEFSELYETLADSDDISALSKEAVESCPLMRFITADTHGYERGSETSTEYERLLSMLNKVKSLKLLNTRRRQLLNLDVLCLSSLIKQSKLKGSKNDKHWVGCCYGSVNDRLVSFHSTKEEFIRLLRNRRKSKAYRKVSLEDLFRTSINEFILKVQRCLSVVGLSFGHYGLSEHLEHECHIPFIEFENFMRSGTHPIMYYTKFEDYDFQPNTEQLRNMHSLKRLSSVCLALTNSMKTSSVARLRQNQLGSVRYQVVECKEVFCQVIKLDSEEYHLLYQKTGESSRCYSIQGPNGHLISFYADPKRFFLPIFSDEVLHNMIDTMISWIRSCPDLKDSIDDVEIALRTLLLLMLTNPTKRNQKQVQNIRYLVMAIVSDFSSTSLMDKLKEDLITPAEKVVYKLLRFLIKTVFGTGEKVLLSAKFKFMLNVSYLCHLITKETPDRLTDQIKCFEKFFEPKSEFGFFVNPKESITPEEECVFYDQMKKFTGKEVDCQRTTPGVNLEMMVSSFNNGTLIFKRLNSLDPMTNSGCATALDLASNKSVVVNKHLNGERLLEYDFNKLLVSAVSQITESFMRKQKYKLNHSDYEYKVSKLVSRLVIGSKETEAGKLEGDSADICFDGEEETSFFKNLEDKVNSTIKRYERSKKTNEGENEVGFENTKGLHHLQTILSGKMAYLRKVILSEISFHLVEDFDPSCLTNDDMKFICEAIETSTELSPLYFTSAVKEQCGLDEMAKNLCRKFFSEGDWFSCMKMILLQMNANAYSGKYRHMQRQGLNFKFDWDKLEEDVRISERESNSESLSKALSLTKCMSAALKNLCFYSEESPTSYTSVGPDSGRLKFALSYKEQVGGNRELYIGDLRTKMFTRLIEDYFESFSSFFSGSCLNNDKEFENAILSMTINVREGLLNYSMDHSKWGPMMCPFLFLMLLQNLKDDQYVRSGKDHISTLLTWHMHKLVEVPFPVVNAMMKSYIKSKLKLLRGSETTVTERIFREYFELGIVPSHISSLIDMGQGILHNASDFYGLISERFINYCIGVIFGERPESYTSSDDQITLFDRRLSELVDSDPEEVLVLLEFHSHLSGLLNKFISPKSVVGRFAAEFKSRFYVWGEEVPLLTKFVSAALHNVKCKEPHQLCETIDTIADQAVANGVPVSLVNCIQKRTLDLLKYANFPLDPFLLNTNTDVKDWLDGSRGYRIQRLIEELCPSETKVMRRLVRRLHHKLKNGEFNEEFFLDLFNRDKKEAILQLGNILGLEEDLSQLANINWLNLNELFPLRMVLRQKVVYPSVMTFQEERIPSLIKTLQNKLCSKFTRGAQKLLSEAINKSAFQSCISSGFIGLCKTLGSRCVRNKNRDNLYIRKVLEDLAMDAHVTAIHRHDGIMLYICDRQSHPEAHCDHISLLRPLLWDYICISLSNSFELGVWVLAEPVKGKNEGSSSLKHLNPCDYVARKPESSRLLEDKISLNHVIQSVRRLYPKIYEDQLLPFMSDMSSKNMRWSPRIKFLDLCVLIDINSESLSLISHVVKWKRDEHYTVLFSDLVNSHQRSDSSLVDEFVVSTRDVCKNFLKQVYFESFVREFVATSRTLGSFSWFPHKDMMPSEDGAEALGPFQSFILKVVNKNMERPMFRNDLQFGFGWFSYRLGDIVCNAAMLIKQGLTNPKAFKSLRNLWDYMINNTEGVLEFSITVDFTHNQNNTDCLRKFSLIFLVKCQLQGPGVAEFLSCSHLFKGEVDRRFLDECLHLLRSDSIFKVNDGVFDIRSEEFEDYMEDPLILGDSLELELIGSRKILDGIRSLDFERIGPEWEPVPLTVRMGALFEGRSLVQNIVVKLETKDMRVFLAELEGYGNFDDVLGSLLLHRFRTGEHLQGSEISTILQELCIDRSILLVPLSLVPDWFTFKDCRLCFSKSKNTVMYETVVGKYRLKGKSCDDWLTKSVVEEID

SEQ ID NO: 9 - protein, 90 aa, Lymphocytic choriomeningitis virus (LCMV)
  amino acid sequence of the Z protein of the MP strain of LCMV
MGQGKSKEGRDASNTSRAEILPDTTYLGPLNCKSCWQRFDSLVRCHDHYLCRHCLNLLLSVSDRCPLCKHPLPTKLKISTAPSSPPPYEE

SEQ ID NO: 10 - DNA, 4604 bp, Lymphocytic choriomeningitis virus (LCMV)
  LCMV clone 13 S-Segment encoding HCMV strain Merlin gB (full-length wildtype)
gcgcaccggggatcctaggctttttggattgcgctttcctctagatcaactgggtgtcaggccctatcctacagaaggatggaatccaggatctggtgcctggtagtctgcgttaacttgtgtatcgtctgtctgggtgctgcggtttcctcatcttctactcgtggaacttctgctactcacagtcaccattcctctcatacgacgtctgctgctcactctcgatccggttcagtctctcaacgcgtaacttcttcccaaacggtcagccatggtgttaacgagaccatctacaacactaccctcaagtacggagatgtggtgggggtcaataccaccaagtacccctatcgcgtgtgttctatggcccagggtacggatcttattcgctttgaacgtaatatcgtctgcacctcgatgaagcccatcaatgaagacctggacgagggcatcatggtggtctacaaacgcaacatcgtcgcgcacacctttaaggtacgagtctaccagaaggttttgacgtttcgtcgtagctacgcttacatccacaccacttatctgctgggcagcaacacggaatacgtggcgcctcctatgtgggagattcatcatatcaacagccacagtcagtgctacagttcctacagccgcgttatagcaggcacggttttcgtggcttatcatagggacagctatgaaaacaaaaccatgcaattaatgcccgacgattattccaacacccacagtacccgttacgtgacggtcaaggatcaatggcacagccgcggcagcacctggctctatcgtgagacctgtaatctgaattgtatggtgaccatcactactgcgcgctccaaatatccttatcattttttcgccacttccacgggtgacgtggttgacatttctcctttctacaacggaaccaatcgcaatgccagctactttggagaaaacgccgacaagtttttcatttttccgaactacactattgtctccgactttggaagaccgaattctgcgttagagacccacaggttggtggcttttcttgaacgtgcggactcggtgatctcctgggatatacaggacgaaaagaatgtcacttgtcaactcactttctgggaagcctcggaacgcaccattcgttccgaagccgaggactcgtatcacttttcttctgccaaaatgaccgccactttcttatctaagaagcaagaggtgaacatgtccgactctgcgctggactgcgtacgtgatgaggctataaataagttacagcagattttcaatacttcatacaatcaaacatatgaaaaatatggaaacgtgtccgtctttgaaaccactggtggtttggtagtgttctggcaaggtatcaagcaaaaatctctggtggaactcgaacgtttggccaaccgctccagtctgaatcttactcataatagaaccaaaagaagtacagatggcaacaatgcaactcatttatccaacatggaatcggtgcacaatctggtctacgcccagctgcagttcacctatgacacgttgcgcggttacatcaaccgggcgctggcgcaaatcgcagaagcctggtgtgtggatcaacggcgcaccctagaggtcttcaaggaactcagcaagatcaacccgtcagccattctctcggccatttacaacaaaccgattgccgcgcgtttcatgggtgatgtcttgggcctggccagctgcgtgaccatcaaccaaaccagcgtcaaggtgctgcgtgatatgaacgtgaaggagtcgccaggacgctgctactcacgacccgtggtcatctttaatttcgccaacagctcgtacgtgcagtacggtcaactgggcgaggacaacgaaatcctgttgggcaaccaccgcactgaggaatgtcagcttcccagcctcaagatcttcatcgccgggaactcggcctacgagtacgtggactacctcttcaaacgcatgattgacctcagcagtatctccaccgtcgacagcatgatcgccctggatatcgacccgctggaaaataccgacttcagggtactggaactttactcgcagaaagagctgcgttccagcaacgtttttgacctcgaagagatcatgcgcgaattcaactcgtacaagcagcgggtaaagtacgtggaggacaaggtagtcgacccgctaccgccctacctcaagggtctggacgacctcatgagcggcctgggcgccgcgggaaaggccgttggcgtagccattggggccgtgggtggcgcggtggcctccgtggtcgaaggcgttgccaccttcctcaaaaaccccttcggagcgttcaccatcatcctcgtggccatagctgtagtcattatcacttatttgatctatactcgacagcggcgtttgtgcacgcagccgctgcagaacctctttccctatctggtgtccgccgacgggaccaccgtgacgtcgggcagcaccaaagacacgtcgttacaggctccgccttcctacgaggaaagtgtttataattctggtcgcaaaggaccgggaccaccgtcgtctgatgcatccacggcggctccgccttacaccaacgagcaggcttaccagatgcttctggccctggcccgtctggacgcagagcagcgagcgcagcagaacggtacagattctttggacggacggactggcacgcaggacaagggacagaagcccaacctactagaccgactgcgacatcgcaaaaacggctaccgacacttgaaagactctgacgaagaagagaacgtctgaagaacagcgcctccctgactctccacctcgaaagaggtggagagtcagggaggcccagagggtcttagagtgtcacaacatttgggcctctaaaaattaggtcatgtggcagaatgttgtgaacagttttcagatctgggagccttgctttggaggcgctttcaaaaatgatgcagtccatgagtgcacagtgcggggtgatctctttcttctttttgtcccttactattccagtatgcatcttacacaaccagccatatttgtcccacactttatcttcatactccctcgaagcttccctggtcatttcaacatcgataagcttaatgtccttcctattttgtgagtccagaagctttctgatgtcatcggagccttgacagcttagaaccatcccctgcggaagagcacctataactgacgaggtcaacccgggttgcgcattgaagaggtcggcaagatccatgccgtgtgagtacttggaatcttgcttgaattgtttttgatcaacgggttccctgtaaaagtgtatgaactgcccgttctgtggttggaaaattgctatttccactggatcattaaatctaccctcaatgtcaatccatgtaggagcgttggggtcaattcctcccatgaggtcttttaaaagcattgtctggctgtagcttaagcccacctgaggtggacctgctgctccaggcgctggcctgggtgagttgactgcaggtttctcgcttgtgagatcaattgttgtgttttcccatgctctccccacaatcgatgttctacaagctatgtatggccatccttcacctgaaaggcaaactttatagaggatgttttcataagggttcctgtccccaacttggtctgaaacaaacatgttgagttttctcttggccccgagaactgccttcaagagatcctcgctgttgcttggcttgatcaaaattgactctaacatgttacccccatccaacagggctgcccctgccttcacggcagcaccaagactaaagttatagccagaaatgttgatgctggactgctgttcagtgatgacccccagaactgggtgcttgtctttcagcctttcaagatcattaagatttggatacttgactgtgtaaagcaagccaaggtctgtgagcgcttgtacaacgtcattgagcggagtctgtgactgtttggccatacaagccatagttagacttggcattgtgccaaattgattgttcaaaagtgatgagtctttcacatcccaaactcttaccacaccacttgcaccctgctgaggctttctcatcccaactatctgtaggatctgagatctttggtctagttgctgtgttgttaagttccccatatatacccctgaagcctggggcctttcagacctcatgatcttggccttcagcttctcaaggtcagccgcaagagacatcagttcttctgcactgagcctccccactttcaaaacattcttctttgatgttgactttaaatccacaagagaatgtacagtctggttgagacttctgagtctctgtaggtctttgtcatctctcttttccttcctcatgatcctctgaacattgctgacctcagagaagtccaacccattcagaaggttggttgcatccttaatgacagcagccttcacatctgatgtgaagctctgcaattctcttctcaatgcttgcgtccattggaagctcttaacttccttagacaaggacatcttgttgctcaatggtttctcaagacaaatgcgcaatcaaatgcctaggatccactgtgcg

SEQ ID NO: 11 - DNA, 35 bp, Artificial Sequence
  WE-specific primer
aatcgtctctaaggatgggtcagattgtgacaatg

SEQ ID NO: 12 - DNA, 35 bp, Artificial Sequence; identical to SEQ ID NO: 11
  WE specific fusion-primer carrying an overhang complementary to the WET-specific primer

SEQ ID NO: 13 - DNA, 37 bp, Artificial Sequence
  WET-specific primer
ctcggtgatcatgttatctgcttcttgttcgatttga

SEQ ID NO: 14 - DNA, 34 bp, Artificial Sequence
  WET-specific fusion-primer complementary to the WE-sequence
aatcgtctctttctttatctcctcttccagatgg

SEQ ID NO: 15 - DNA, 23 bp, Artificial Sequence
  Primer specific for LCMV NP
ggctcccagatctgaaaactgtt

SEQ ID NO: 16 - DNA, 22 bp, Artificial Sequence
  NP- and GP-specific primer
gctggcttgtcactaatggctc

SEQ ID NO: 17 - DNA, 535 bp, Artificial Sequence
  Representative cDNA sequence obtained from animal #3 (r3LCMV-GFPnat #3) revealing a recombined S segment combining NP and GP sequences
aagaagcagataacatgatcaccgagatgctgaggaaggactacatcaagagacagggcagcacccccctggccctcatggatctgctcatgttcagcaccagcgcctacctcatcagcatcttcctgcacctggtgaagatccccacccacagacacatcaagggcggcagctgccccaagccccacagactcaccaacaagggcatctgcagctgcggcgccttcaaggtgcccggcgtaaaaaccatctggaagaggagataaagaacagcgcctccctgactctccacctcgaaagaggtggagagtcagggaggcccagagggtcttacttgtacagctcgtccatgccgagagtgatcccggcggcggtcacgaactccagcaggaagaacagcgcctccctgactctccacctcgaaagaggtggagagtcagggaggcccagaggtcttagagtgtcacaacatttgggcctctaaaaattaggtcatgtggcagaatgttgtgaacagttttcagatctgggagcc

SEQ ID NO: 18 - DNA, 2555 bp, Artificial Sequence
  S segment 1 of r3LCMV-P1A (containing NP)
gcgcaccggggatcctaggctttttggattgcgctttcctctagatcaactgggtgtcaggccctatcctacagaaggatgagcgacaacaagaagcccgacaaggcccactctggcagcggcggagatggcgacggcaacagatgtaacctgctgcacagatacagcctggaagagatcctgccctacctgggctggctggtgttcgccgtcgtgacaacaagcttcctggccctgcagatgttcatcgacgccctgtacgaggaacagtacgagagggacgtggcctggatcgccagacagagcaagagaatgagcagcgtggacgaggacgaggatgatgaggacgacgaagatgactactacgacgatgaggatgacgacgacgacgccttctacgatgacgaggacgatgaagaggaagaactggaaaacctgatggacgacgagtccgaggatgaggccgaggaagagatgagcgtggaaatgggcgctggcgccgaagagatgggagccggcgctaactgtgcttgcgtgccaggacaccacctgagaaagaacgaagtgaagtgccggatgatctacttcttccacgaccccaactttctggtgtccatccccgtgaaccccaaagaacagatggaatgcagatgcgagaacgccgacgaagaggtggccatggaagaagaagaggaagaggaagaagaagaagaagaggaagaaatgggcaaccccgacggcttcagcccctgaagaacagcgcctccctgactctccacctcgaaagaggtggagagtcagggaggcccagagggtcttagagtgtcacaacatttgggcctctaaaaattaggtcatgtggcagaatgttgtgaacagttttcagatctgggagccttgctttggaggcgctttcaaaaatgatgcagtccatgagtgcacagtgcggggtgatctctttcttctttttgtcccttactattccagtatgcatcttacacaaccagccatatttgtcccacactttatcttcatactccctcgaagcttccctggtcatttcaacatcgataagcttaatgtccttcctattttgtgagtccagaagctttctgatgtcatcggagccttgacagcttagaaccatcccctgcggaagagcacctataactgacgaggtcaacccgggttgcgcattgaagaggtcggcaagatccatgccgtgtgagtacttggaatcttgcttgaattgtttttgatcaacgggttccctgtaaaagtgtatgaactgcccgttctgtggttggaaaattgctatttccactggatcattaaatctaccctcaatgtcaatccatgtaggagcgttggggtcaattcctcccatgaggtcttttaaaagcattgtctggctgtagcttaagcccacctgaggtggacctgctgctccaggcgctggcctgggtgagttgactgcaggtttctcgcttgtgagatcaattgttgtgttttcccatgctctccccacaatcgatgttctacaagctatgtatggccatccttcacctgaaaggcaaactttatagaggatgttttcataagggttcctgtccccaacttggtctgaaacaaacatgttgagttttctcttggccccgagaactgccttcaagagatcctcgctgttgcttggcttgatcaaaattgactctaacatgttacccccatccaacagggctgcccctgccttcacggcagcaccaagactaaagttatagccagaaatgttgatgctggactgctgttcagtgatgacccccagaactgggtgcttgtctttcagcctttcaagatcattaagatttggatacttgactgtgtaaagcaagccaaggtctgtgagcgcttgtacaacgtcattgagcggagtctgtgactgtttggccatacaagccatagttagacttggcattgtgccaaattgattgttcaaaagtgatgagtctttcacatcccaaactcttaccacaccacttgcaccctgctgaggctttctcatcccaactatctgtaggatctgagatctttggtctagttgctgtgttgttaagttccccatatatacccctgaagcctggggcctttcagacctcatgatcttggccttcagcttctcaaggtcagccgcaagagacatcagttcttctgcactgagcctccccactttcaaaacattcttctttgatgttgactttaaatccacaagagaatgtacagtctggttgagacttctgagtctctgtaggtctttgtcatctctcttttccttcctcatgatcctctgaacattgctgacctcagagaagtccaacccattcagaaggttggttgcatccttaatgacagcagccttcacatctgatgtgaagctctgcaattctcttctcaatgcttgcgtccattggaagctcttaacttccttagacaaggacatcttgttgctcaatggtttctcaagacaaatgcgcaatcaaatgcctaggatccactgtgcg

SEQ ID NO: 19 - DNA, 2375 bp, Artificial Sequence
  S segment 2 of r3LCMV-P1A (containing GP)
gcgcaccggggatcctaggctttttggattgcgctttcctctagatcaactgggtgtcaggccctatcctacagaaggatgagcgacaacaagaagcccgacaaggcccactctggcagcggcggagatggcgacggcaacagatgtaacctgctgcacagatacagcctggaagagatcctgccctacctgggctggctggtgttcgccgtcgtgacaacaagcttcctggccctgcagatgttcatcgacgccctgtacgaggaacagtacgagagggacgtggcctggatcgccagacagagcaagagaatgagcagcgtggacgaggacgaggatgatgaggacgacgaagatgactactacgacgatgaggatgacgacgacgacgccttctacgatgacgaggacgatgaagaggaagaactggaaaacctgatggacgacgagtccgaggatgaggccgaggaagagatgagcgtggaaatgggcgctggcgccgaagagatgggagccggcgctaactgtgcttgcgtgccaggacaccacctgagaaagaacgaagtgaagtgccggatgatctacttcttccacgaccccaactttctggtgtccatccccgtgaaccccaaagaacagatggaatgcagatgcgagaacgccgacgaagaggtggccatggaagaagaagaggaagaggaagaagaagaagaagaggaagaaatgggcaaccccgacggcttcagcccctgaagaacagcgcctccctgactctccacctcgaaagaggtggagagtcagggaggcccagagggtctcagcgtcttttccagacggtttttacaccaggcaccttaaatgcaccacaactacaaattcctttgttggttaatcggtgtggctttggacatgagccaccttttatgtgcctgtgtgttggtattttgacaaggtgcaggaagatgctgactagatatgcagatgtggaaaacatcagaaggtccatcaatgctaggggggtactcccctgcctctttatgtaatccttcctcaacatctctgtaatcatgttatcggcttcctgttcgatttggtcactgaagtgggtctcatttaagtaagaaccattggtgacaagccagcacttggggacactagtttcgccggtctttgcatgttctaggtaccaaaactttgagtaattgcaatatggcacccccatcagatctctcaagtggttcctcatcagtagttgatctgaaatcaaagaattcactgttgttttgaataagtgcaaggcagattctacgtcctctttgaacttactcaaagcagccttgttgtagtcaattagtcgcagcatgtcacagaattcttcatcatgatttacattgcatttcgcaactgctgtgttcccgaaacacttaagctctgcagcaagaatcatccatttggtcaggcaataaccacctggattctccacccctgaagagtctgacaaagtccaggtgaatgtgcccgctagtctcctagtggagaacttagttttctcttgggaaaggagaatcctggacatcccaaaaggacctgcatatgtgcagtggttttcccaggttctattttgtataatcaggtattggtaactcgtctggctacaccaggtggtcttgccatctgagcctgtccagccccagccactcctcatgtatttccccccgaaggcagttctaaacatatctaggactctacctctgaaggttctacactggctctgagcactttgtgcatctgagaatgtcaagttgtattggatggttatgccattgttgaagtcgcaggatactgccttatagttggagttccctctgatactgaggtgtaggctcgaaactatactcatgagtgtgtggtcaaaggtctttttgttgaaggcagaggtcagattgcaaaagttgtgactgatgatggaatcattggtgaaggtcaattctagtccagaagtccccatactgatgtaatggtgggagttgttggctgaacatgcgttgggcatggtcaggttcagatgtgacatatcaaactccactgacttaaattggtaaactcctttgtaaatgtcgggtcccttaagaccgtacatgccacaggacctgccagccagaagtaggaaactgatcaatgcgaatatcccacaggtggcaaaattgtagacagccttgatacccgtgatcacgataagcacaataatgacaatgttgatcacctcatcgatgatgtgaggcagagcctcaaacattgtcacaatctgacccatcttgttgctcaatggtttctcaagacaaatgcgcaatcaaatgcctaggatccactgtgcg

SEQ ID NO: 20 - DNA, 7229 bp, Artificial Sequence; identical to SEQ ID NO: 3
  L segment of r3LCMV-P1A

SEQ ID NO: 21 - DNA, 2628 bp, Artificial Sequence
  S segment 1 of r3JUNV-P1A (containing NP)
gcgcaccggggatcctaggcgattttggttacgctataattgtaactgttttctgtttggacaacatcaaaaacatccattgcacaatgagcgacaacaagaagcccgacaaggcccactctggcagcggcggagatggcgacggcaacagatgtaacctgctgcacagatacagcctggaagagatcctgccctacctgggctggctggtgttcgccgtcgtgacaacaagcttcctggccctgcagatgttcatcgacgccctgtacgaggaacagtacgagagggacgtggcctggatcgccagacagagcaagagaatgagcagcgtggacgaggacgaggatgatgaggacgacgaagatgactactacgacgatgaggatgacgacgacgacgccttctacgatgacgaggacgatgaagaggaagaactggaaaacctgatggacgacgagtccgaggatgaggccgaggaagagatgagcgtggaaatgggcgctggcgccgaagagatgggagccggcgctaactgtgcttgcgtgccaggacaccacctgagaaagaacgaagtgaagtgccggatgatctacttcttccacgaccccaactttctggtgtccatccccgtgaaccccaaagaacagatggaatgcagatgcgagaacgccgacgaagaggtggccatggaagaagaagaggaagaggaagaagaagaagaagaggaagaaatgggcaaccccgacggcttcagcccctgagacctcctgagggtccccaccagcccgggcactgcccgggctggtgtggccccccagtccgcggcctggccgcggactggggaggcactgcttacagtgcataggctgccttcgggaggaacagcaagctcggtggtaatagaggtgtaggttcctcctcatagagcttcccatctagcactgactgaaacattatgcagtctagcagagcacagtgtggttcactggaggccaacttgaagggagtatccttttccctctttttcttattgacaaccactccattgtgatatttgcataagtgaccatatttctcccagacctgttgatcaaactgcctggcttgttcagatgtgagcttaacatcaaccagtttaagatctcttcttccatggaggtcaaacaacttcctgatgtcatcggatccttgagtagtcacaaccatgtctggaggcagcaagccgatcacgtaactaagaactcctggcattgcatcttctatgtccttcattaagatgccgtgagagtgtctgctaccatttttaaaccctttctcatcatgtggttttctgaagcagtgaatgtactgcttacctgcaggttggaataatgccatctcaacagggtcagtggctggtccttcaatgtcgagccaaagggtgttggtggggtcgagtttccccactgcctctctgatgacagcttcttgtatctctgtcaagttagccaatctcaaattctgaccgtttttttccggctgtctaggaccagcaactggtttccttgtcagatcaatacttgtgttgtcccatgacctgcctgtgatttgtgatctagaaccaatataaggccaaccatcgccagaaagacaaagtttgtacaaaaggttttcataaggatttctattgcctggtttctcatcaataaacatgccttctcttcgtttaacctgaatggttgattttatgagggaagagaagttttctggggtgactctgattgtttccaacatgtttccaccatcaagaatagatgctccagcctttactgcagctgaaagactgaagttgtaaccagaaatattgatggagctttcatctttagtcacaatctgaaggcagtcatgttcctgagtcagtctgtcaaggtcacttaagtttggatacttcacagtgtatagaagcccaagtgaggttaaagcttgtatgacactgttcattgtctcacctccttgaacagtcatgcatgcaattgtcaatgcaggaacagagccaaactgattgtttagctttgaagggtctttaacatcccatatcctcaccacaccatttcccccagtcccttgctgttgaaatcccagtgttctcaatatctctgatcttttagcaagttgtgactgggacaagttacccatgtaaaccccctgagagcctgtctctgctcttcttatcttgttttttaatttctcaaggtcagacgccaactccatcagttcatccctccccagatctcccaccttgaaaactgtgtttcgttgaacactcctcatggacatgagtctgtcaacctctttattcaggtccctcaacttgttgagatcttcttccccctttttagtctttctgagtgcccgctgcacctgtgccacttggttgaagtcgatgctgtcagcaattagcttggcgtccttcaaaacatctgacttgacagtctgagtgaattggctcaaacctctccttaaggactgagtccatctaaagcttggaacctccttggagtgtgccatgccagaagttctggtgattttgatctagaatagagttgctcagtgaaagtgttagacactatgcctaggatccactgtgcg

SEQ ID NO: 22 - DNA, 2391 bp, Artificial Sequence
  S segment 2 of r3JUNV-P1A (containing GP)
gcgcaccggggatcctaggcgattttggttacgctataattgtaactgttttctgtttggacaacatcaaaaacatccattgcacaatgagcgacaacaagaagcccgacaaggcccactctggcagcggcggagatggcgacggcaacagatgtaacctgctgcacagatacagcctggaagagatcctgccctacctgggctggctggtgttcgccgtcgtgacaacaagcttcctggccctgcagatgttcatcgacgccctgtacgaggaacagtacgagagggacgtggcctggatcgccagacagagcaagagaatgagcagcgtggacgaggacgaggatgatgaggacgacgaagatgactactacgacgatgaggatgacgacgacgacgccttctacgatgacgaggacgatgaagaggaagaactggaaaacctgatggacgacgagtccgaggatgaggccgaggaagagatgagcgtggaaatgggcgctggcgccgaagagatgggagccggcgctaactgtgcttgcgtgccaggacaccacctgagaaagaacgaagtgaagtgccggatgatctacttcttccacgaccccaactttctggtgtccatccccgtgaaccccaaagaacagatggaatgcagatgcgagaacgccgacgaagaggtggccatggaagaagaagaggaagaggaagaagaagaagaagaggaagaaatgggcaaccccgacggcttcagcccctgagacctcctgagggtccccaccagcccgggcactgcccgggctggtgtggccccccagtccgcggcctggccgcggactggggaggcactgcatggggcagttcattagcttcatgcaagaaataccaacctttttgcaggaggctctgaacattgctcttgttgcagtcagtctcattgccatcattaagggtatagtgaacttgtacaaaagtggtttattccaattctttgtattcctagcgcttgcaggaagatcctgcacagaagaagctttcaaaatcggactgcacactgagttccagactgtgtccttctcaatggtgggtctcttttccaacaatccacatgacctacctttgttgtgtaccttaaacaagagccatctttacattaaggggggcaatgcttcatttcagatcagctttgatgatattgcagtattgttgccacagtatgatgttataatacaacatccagcagatatgagctggtgttccaaaagtgatgatcaaatttggttgtctcagtggttcatgaatgctgtgggacatgattggcatctagacccaccatttctgtgtaggaaccgtgcaaagacagaaggcttcatctttcaagtcaacacctccaagactggtgtcaatggaaattatgctaagaagtttaagactggcatgcatcatttatatagagaatatcctgacccttgcttgaatggcaaactgtgcttaatgaaggcacaacctaccagttggcctctccaatgtccactcgaccacgttaacacattacacttccttacaagaggtaaaaacattcaacttccaaggaggtccttgaaagcattcttctcctggtctttgacagactcatccggcaaggatacccctggaggctattgtctagaagagtggatgctcgtagcagccaaaatgaagtgttttggcaatactgctgtagcaaaatgcaatttgaatcatgactctgaattctgtgacatgttgaggctctttgattacaacaaaaatgctatcaaaaccctaaatgatgaaactaagaaacaagtaaatctgatggggcagacaatcaatgccctgatatctgacaatttattgatgaaaaacaaaattagggaactgatgagtgtcccttactgcaattacacaaaattttggtatgtcaaccacacactttcaggacaacactcattaccaaggtgctggttaataaaaaacaacagctatttgaacatctctgacttccgtaatgactggatattagaaagtgacttcttaatttctgaaatgctaagcaaagagtattcggacaggcagggtaaaactcctttgactttagttgacatctgtatttggagcacagtattcttcacagcgtcactcttccttcacttggtgggtataccctcccacagacacatcaggggcgaagcatgccctttgccacacaggttgaacagcttgggtggttgcagatgtggtaagtaccccaatctaaagaaaccaacagtttggcgtagaggacactaagccagaagttctggtgattttgatctagaatagagttgctcagtgaaagtgttagacactatgcctaggatccactgtgcg

SEQ ID NO: 23 - DNA, 7115 bp, Artificial Sequence
  L segment of r3JUNV-P1A
gcgcaccggggatcctaggcgtaacttcatcattaaaatctcagattctgctctgagtgtgacttactgcgaagaggcagacaaatgggcaactgcaacggggcatccaagtctaaccagccagactcctcaagagccacacagccagccgcagaatttaggagggtagctcacagcagtctatatggtagatataactgtaagtgctgctggtttgctgataccaatttgataacctgtaatgatcactacctttgtttaaggtgccatcagggtatgttaaggaattcagatctctgcaatatctgctggaagcccctgcccaccacaatcacagtaccggtggagccaacagcaccaccaccataggcagactgcacagggtcagacccgaccccccggggggcccccatggggaccccccgtgggggaaccccgggggtgatgcgccattagtcaatgtctttgatctcgactttgtgcttcagtggcctgcatgtcacccctttcaatctgaactgcccttggggatctgatatcagcaggtcatttaaagatctgctgaatgccaccttgaaatttgagaattccaaccagtcaccaaatttatcaagtgaacggatcaactgctctttgtgtagatcataaacgaggacaaagtcctcttgctgaaataatattgtttgtgatgttgtttttagataaggccatagttggcttaataaggtttccacactatcaatgtcctctagtgctccaattgccttgactatgacatccccagacaactcaactctatatgttgacaacctttcattacctctgtaaaagataccctctttcaagacaagaggttctcctgggttatctggcccaatgaggtcatatgcatacttgttacttagttcagaataaaagtcaccaaagttgaacttaacatggctcagaatattgtcatcatttgtcgcagcgtagcctgcatcaataaacaagccagctaggtcaaagctctcatggcctgtgaacaatggtaggctagcgataaccagtgcaccatccaacaatgagtggcttccctcagacccagaaacacattgactcattgcatccacattcagctctaattcaggggtaccgacatcatccactcctagtgaactgacaatggtgtaactgtacaccatctttcttctaagtttaaattttgtcgaaactcgtgtgtgttctacttgaatgatcaattttagtttcacagcttcttggcaagcaacattgcgcaacacagtgtgcaggtccatcatgtcttcctgaggcaacaaggagatgttgtcaacagagacaccctcaaggaaaaccttgatattatcaaagctagaaactacataacccattgcaatgtcttcaacaaacattgctcttgatactttattattcctaactgacaaggtaaaatctgtgagttcagctagatctacttgactgtcatcttctagatctagaacttcattgaaccaaaagaaggatttgagacacgatgttgacatgactagtgggtttatcatcgaagataagacaacttgcaccatgaagttcctgcaaacttgctgtgggctgatgccaacttcccaatttgtatactctgactgtctaacatgggctgaagcgcaatcactctgtttcacaatataaacattattatctcttactttcaataagtgacttataatccctaagttttcattcatcatgtctagagccacacagacatctagaaacttgagtcttccactatccaaagatctgttcacttgaagatcattcataaagggtgccaaatgttcttcaaatagtttggggtaatttcttcgtatagaatgcaatacatggttcatgcctaattggtcttctatctgtcgtactgctttgggtttaacagcccagaagaaattcttattacataagaccagaggggcctgtggactcttaatagcagaaaacacccactcccctaactcacaggcatttgtcagcaccaaagagaagtaatcccacaaaattggtttagaaaattggttaacttctttaagtgatttttgacagtaaataactttaggctttctctcacaaattccacaaagacatggcattattcgagtaaatatgtcctttatatacagaaatccgcctttaccatccctaacacacttactccccatactcttacaaaacccaatgaagcctgaggcaacagaagactgaaatgcagatttgttgattgactctgccaagatcttcttcacgccttttgtgaaatttcttgacagcctggactgtattgtccttatcaatgttggcatctcttctttctctaacactcttcgacttgtcatgagtttggtcctcaagaccaacctcaagtccccaaagctcgctaaattgacccatctgtagtctagagtttgtctgatttcatcttcactacacccggcatattgcaggaatccggataaagcctcatcccctcccctgcttatcaagttgataaggttttcctcaaagattttgcctctcttaatgtcattgaacactttcctcgcgcagttccttataaacattgtctccttatcatcagaaaaaatagcttcaattttcctctgtagacggtaccctctagacccatcaacccagtctttgacatcttgttcttcaatagctccaaacggagtctctctgtatccagagtatctaatcaattggttgactctaatggaaatctttgacactatatgagtgctaaccccattagcaatacattgatcacaaattgtgtctatggtctctgacagttgtgttggagttttacacttaacgttgtgtagagcagcagacacaaacttggtgagtaaaggagtctcttcacccatgacaaaaaatcttgacttaaactcagcaacaaaagttcctatcacactctttgggctgataaacttgtttaatttagaagataagaattcatggaagcacaccatttccagcagttctgtcctgtcttgaaacttttcatcactaaggcaaggaatttttataaggctaacctggtcatcgctggaggtataagtgacaggtatcacatcatacaataagtcaagtgcataacacagaaattgttcagtaattagcccatataaatctgatgtgttgtgcaagattccctggcccatgtccaagacagacattatatggctggggacctggtcccttgactgcagatactggtgaaaaaactcttcaccaacactagtacagtcacaacccattaaacctaaagatctcttcaatttccctacacagtaggcttctgcaacattaattggaacttcaacgaccttatgaagatgccatttgagaatgttcattactggttcaagattcacctttgttctatctctgggattcttcaattctaatgtgtacaaaaaagaaaggaaaagtgctgggctcatagttggtccccatttggagtggtcatatgaacaggacaagtcaccattgttaacagccattttcatatcacagattgcacgttcgaattccttttctgaattcaagcatgtgtatttcattgaactacccacagcttctgagaagtcttcaactaacctggtcatcagcttagtgttgaggtctcccacatacagttctctatttgagccaacctgctccttataacttagtccaaatttcaagttccctgtatttgagctgatgcttgtgaactctgtaggagagtcgtctgaatagaaacataaattccgtagggctgcatttgtaaaataacttttgtctagcttatcagcaatggcttcagaattgctttccctggtactaagccgaacctcatcctttagtctcagaacttcactggaaaagcccaatctagatctacttctatgctcataactacccaatttctgatcataatgtccttgaattaaaagatacttgaagcattcaaagaattcatcttcttggtaggctattgttgtcaaattttttaataacaaacccaaagggcagatgtcctgcggtgcttcaagaaaataagtcaatttaaatggagatagataaacagcatcacataactctttatacacatcagacctgagcacatctggatcaaaatccttcacctcatgcattgacacctctgctttaatctctctcaacactccaaaaggggcccacaatgactcaagagactctcgctcatcaacagatggattttttgatttcaacttggtgatctcaacttttgtcccctcactattagccatcttggctagtgtcatttgtacgtcatttctaataccctcaaaggcccttacttgatcctctgttaaactctcatacatcactgataattcttcttgattggttctggttcttgaaccggtgctcacaagacctgttagattttttaatattaagtagtccatggaatcaggatcaagattatacctgccttttgttttaaacctctcagccatagtagaaacgcatgttgaaacaagtttctccttatcataaacagaaagaatatttccaagttcgtcgagcttggggattaccacacttttattgcttgacagatccagagctgtgctagtgatgttaggcctgtagggattgcttttcagttcacctgtaactttaagtcttcctctattgaagagagaaatgcagaaggacaaaatctctttacacactcctggaatttgagtatctgaggaagtcttagcctctttggaaaagaatctgtccaatcctcttatcatggtgtcctcttgttccagtgttagactcccacttagaggggggtttacaacaacacaatcaaacttgactttgggctcaataaacttctcaaaacactttatttgatctgtcaggcgatcaggtgtctctttggttaccaagtgacacagataactaacatttaatagatatttaaaccttcttgcaaagtaaagatctgcatcttccccttcacccaaaattgtctggaaaagttccacagccatcctctgaatcagcacctctgatccagacatgcagtcgacccttaactttgacatcaaatccacatgatggatttgatttgcatatgccatcaagaaatatcttagaccttgtaaaaatgtctggttccttttggaaggggaacagagtacagctaacactaacaatcttaatattggccttgtcattgtcatgagttcgtggctaaaatccaaccagctggtcatttcctcacacatttcaattaacacatcctccgaaaatataggcaggaaaaatctctttggatcacagtaaaaagagccttgttcttccaataccccattgatggatagatagatagaatagcaccttgacttctcacctgttttttggtaaaacaagagaccaaatgtattctttgtcagatgaaatctttgtacataacactctcttagtctaacattcccaaaatatctagaatactctctttcattgattaacaatcgggaggaaaatgatgtcttcatcgagttgaccaatgcaagggaaatggaggacaaaatcctaaataatttcttctgctcaccttccactaagctgctgaatggctgatgtctacagattttctcaaattccttgttaatagtatatctcatcactggtctgtcagaaacaagtgcctgagctaaaatcatcaagctatccatatcagggtgttttattagtttttccagctgtgaccagagatcttgatgagagttcttcaatgttctggaacacgcttgaacccacttggggctggtcatcaatttcttccttattagtttaatcgcctccagaatatctagaagtctgtcattgactaacattaacatttgtccaacaactattcccgcatttcttaaccttacaattgcatcatcatgcgttttgaaaagatcacaaagtaaattgagtaaaactaagtccagaaacagtaaagtgtttctcctggtgttgaaaacttttagacctttcactttgttacacacggaaagggcttgaagataacacctctctacagcatcaatagatatagaattctcatctgactggctttccatgttgacttcatctattggatgcaatgcgatagagtagactacatccatcaacttgtttgcacaaaaagggcagctgggcacatcactgtctttgtggcttcctaataagatcaagtcatttataagcttagacttttgtgaaaatttgaatttccccaactgcttgtcaaaaatctccttcttaaaccaaaaccttaactttatgagttcttctcttatgacagattctctaatgtctcctctaaccccaacaaagagggattcatttaacctctcatcataacccaaagaattctttttcaagcattcgatgttttctaatcccaagctctggttttttgtgttggacaaactatggatcaatcgctggtattcttgttcttcaatattaatctcttgcataaattttgatttctttaggatgtcgatcagcaaccaccgaactctttcaacaacccaatcagcaaggaatctattgctgtagctagatctgccatcaaccacaggaaccaacgtaatccctgcccttagtaggtcggactttaggtttaagagctttgacatgtcactcttccattttctctcaaactcatcaggattgaccctaacaaaggtttccaataggatgagtgttttccctgtgagtttgaagccatccggaatgacttttggaagggtgggacatagtatgccatagtcagacaggatcacatcaacaaacttctgatctgaattgatctgacaggcgtgtgcctcacaggactcaagctctactaaacttgacagaagtttgaacccttccaacaacagagagctggggtgatgttgagataaaaagatgtccctttggtatgctagctcctgtctttctggaaaatgctttctaataaggctttttatttcatttactgattcctccatgctcaagtgccgcctaggatcctcggtgcg

SEQ ID NO: 24 - protein, 224 aa, Artificial Sequence
  Amino acid sequence of a P815 mouse mastocytoma-derived self antigen P1A
MSDNKKPDKAHSGSGGDGDGNRCNLLHRYSLEEILPYLGWLVFAVVTTSFLALQMFIDALYEEQYERDVAWIARQSKRMSSVDEDEDDEDDEDDYYDDEDDDDDAFYDDEDDEEEELENLMDDESEDEAEEEMSVEMGAGAEEMGAGANCACVPGHHLRKNEVKCRMIYFFHDPNFLVSIPVNPKEQMECRCENADEEVAMEEEEEEEEEEEEEEMGNPDGFSP